European Patent Specification EP 3 808 365 B1, published January 31, 2024. Title: DELIVERY OF THERAPEUTIC AGENTS BY A COLLAGEN BINDING PROTEIN. Applicant: THE BOARD OF TRUSTEES OF THE UNIVERSITY OF ARKANSAS MONTEFIORE MEDICAL CENTER KITASATO UNIVERSITY GENSURE, Robert C. PONNAPAKKAM, Tulasi KATIKANENI, Ranjitha PHILOMINATHAN, Sagaya Theresa Leena KOIDE, Takaki MATSUSHITA, Osamu SAKON, Joshua. The sequence listing filed with the application follows.

SEQUENCE LISTING (47 sequences)

SEQ ID NO: 1 - protein, 158 aa, Artificial Sequence
  Synthetic fusion protein containing parathyroid hormone segment and collagen-binding domain
SVSEIQLMHNLGKHLNSMERVEWLRKKLQDVHNGINSPVYPIGTEKEPNNSKETASGPIVPGIPVSGTIENTSDQDYFYFDVITPGEVKIDINKLGYGGATWVVYDENNNAVSYATDDGQNLSGKFKADKPGRYYIHLYMFNGSYMPYRINIEGSVGR

SEQ ID NO: 2 - protein, 251 aa, Artificial Sequence
  Synthetic fusion protein containing parathyroid hormone fragment and collagen-binding domain and polycystic kidney disease domain of ColH.
SVSEIQLMHNLGKHLNSMERVEWLRKKLQDVHNGIPEIKDLSENKLPVIYMHVPKSGALNQKVVFYGKGTYDPDGSIAGYQWDFGDGSDFSSEQNPSHVYTKKGEYTVTLRVMDSSGQMSEKTMKIKITDPVYPIGTEKEPNNSKETASGPIVPGIPVSGTIENTSDQDYFYFDVITPGEVKIDINKLGYGGATWVVYDENNNAVSYATDDGQNLSGKFKADKPGRYYIHLYMFNGSYMPYRINIEGSVGR

SEQ ID NO: 3 - DNA, 5464 bp, Artificial Sequence
  Synthetic expression vector
agcttatcgactgcacggtgcaccaatgcttctggcgtcaggcagccatcggaagctgtggtatggctgtgcaggtcgtaaatcactgcataattcgtgtcgctcaaggcgcactcccgttctggataatgttttttgcgccgacatcataacggttctggcaaatattctgaaatgagctgttgacaattaatcatcggctcgtataatgtgtggaattgtgagcggataacaatttcacacaggaaacagtattcatgtcccctatactaggttattggaaaattaagggccttgtgcaacccactcgacttcttttggaatatcttgaagaaaaatatgaagagcatttgtatgagcgcgatgaaggtgataaatggcgaaacaaaaagtttgaattgggtttggagtttcccaatcttccttattatattgatggtgatgttaaattaacacagtctatggccatcatacgttatatagctgacaagcacaacatgttgggtggttgtccaaaagagcgtgcagagatttcaatgcttgaaggagcggttttggatattagatacggtgtttcgagaattgcatatagtaaagactttgaaactctcaaagttgattttcttagcaagctacctgaaatgctgaaaatgttcgaagatcgtttatgtcataaaacatatttaaatggtgatcatgtaacccatcctgacttcatgttgtatgacgctcttgatgttgttttatacatggacccaatgtgcctggatgcgttcccaaaattagtttgttttaaaaaacgtattgaagctatcccacaaattgataagtacttgaaatccagcaagtatatagcatggcctttgcagggctggcaagccacgtttggtggtggcgaccatcctccaaaatcggatctgatcgaaggtcgttctgtgagtgaaatacagcttatgcataacctgggaaaacatctgaactcgatggagagagtagaatggctgcgtaagaagctgcaggatgtgcacaatggaattaattccccggtatatccaataggcactgaaaaagaaccaaataacagtaaagaaactgcaagtggtccaatagtaccaggtatacctgttagtggaaccatagaaaatacaagtgatcaagattatttctattttgatgttataacaccaggagaagtaaaaatagatataaataaattagggtacggaggagctacttgggtagtatatgatgaaaataataatgcagtatcttatgccactgatgatgggcaaaatttaagtggaaagtttaaggcagataaaccaggtagatattacatccatctttacatgtttaatggtagttatatgccatatagaattaatatagaaggttcagtaggaagataatattttattagttgaggtaactccactcgaattggtcgactcgagcggccgcatcgtgactgactgacgatctgcctcgcgcgtttcggtgatgacggtgaaaacctctgacacatgcagctcccggagacggtcacagcttgtctgtaagcggatgccgggagcagacaagcccgtcagggcgcgtcagcgggtgttggcgggtgtcggggcgcagccatgacccagtcacgtagcgatagcggagtgtataattcttgaagacgaaagggcctcgtgatacgcctatttttataggttaatgtcatgataataatggtttcttagacgtcaggtggcacttttcggggaaatgtgcgcggaacccctatttgtttatttttctaaatacattcaaatatgtatccgctcatgagacaataaccctgataaatgcttcaataatattgaaaaaggaagagtatgagtattcaacatttccgtgtcgcccttattcccttttttgcggcattttgccttcctgtttttgctcacccagaaacgctggtgaaagtaaaagatgctgaagatcagttgggtgcacgagtgggttacatcgaactggatctcaacagcggtaagatccttgagagttttcgccccgaagaacgttttccaatgatgagcacttttaaagttctgctatgtggcgcggtattatcccgtgttgacgccgggcaagagcaactcggtcgccgcatacactattctcagaatgacttggttgagtactcaccagtcacagaaaagcatcttacggatggcatgacagtaagagaattatgcagtgctgccataaccatgagtgataacactgcggccaacttacttctgacaacgatcggaggaccgaaggagctaaccgcttttttgcacaacatgggggatcatgtaactcgccttgatcgttgggaaccggagctgaatgaagccataccaaacgacgagcgtgacaccacgatgcctgcagcaatggcaacaacgttgcgcaaactattaactggcgaactacttactctagcttcccggcaacaattaatagactggatggaggcggataaagttgcaggaccacttctgcgctcggcccttccggctggctggtttattgctgataaatctggagccggtgagcgtgggtctcgcggtatcattgcagcactggggccagatggtaagccctcccgtatcgtagttatctacacgacggggagtcaggcaactatggatgaacgaaatagacagatcgctgagataggtgcctcactgattaagcattggtaactgtcagaccaagtttactcatatatactttagattgatttaaaacttcatttttaatttaaaaggatctaggtgaagatcctttttgataatctcatgaccaaaatcccttaacgtgagttttcgttccactgagcgtcagaccccgtagaaaagatcaaaggatcttcttgagatcctttttttctgcgcgtaatctgctgcttgcaaacaaaaaaaccaccgctaccagcggtggtttgtttgccggatcaagagctaccaactctttttccgaaggtaactggcttcagcagagcgcagataccaaatactgtccttctagtgtagccgtagttaggccaccacttcaagaactctgtagcaccgcctacatacctcgctctgctaatcctgttaccagtggctgctgccagtggcgataagtcgtgtcttaccgggttggactcaagacgatagttaccggataaggcgcagcggtcgggctgaacggggggttcgtgcacacagcccagcttggagcgaacgacctacaccgaactgagatacctacagcgtgagctatgagaaagcgccacgcttcccgaagggagaaaggcggacaggtatccggtaagcggcagggtcggaacaggagagcgcacgagggagcttccagggggaaacgcctggtatctttatagtcctgtcgggtttcgccacctctgacttgagcgtcgatttttgtgatgctcgtcaggggggcggagcctatggaaaaacgccagcaacgcggcctttttacggttcctggccttttgctggccttttgctcacatgttctttcctgcgttatcccctgattctgtggataaccgtattaccgcctttgagtgagctgataccgctcgccgcagccgaacgaccgagcgcagcgagtcagtgagcgaggaagcggaagagcgcctgatgcggtattttctccttacgcatctgtgcggtatttcacaccgcataaattccgacaccatcgaatggtgcaaaacctttcgcggtatggcatgatagcgcccggaagagagtcaattcagggtggtgaatgtgaaaccagtaacgttatacgatgtcgcagagtatgccggtgtctcttatcagaccgtttcccgcgtggtgaaccaggccagccacgtttctgcgaaaacgcgggaaaaagtggaagcggcgatggcggagctgaattacattcccaaccgcgtggcacaacaactggcgggcaaacagtcgttgctgattggcgttgccacctccagtctggccctgcacgcgccgtcgcaaattgtcgcggcgattaaatctcgcgccgatcaactgggtgccagcgtggtggtgtcgatggtagaacgaagcggcgtcgaagcctgtaaagcggcggtgcacaatcttctcgcgcaacgcgtcagtgggctgatcattaactatccgctggatgaccaggatgccattgctgtggaagctgcctgcactaatgttccggcgttatttcttgatgtctctgaccagacacccatcaacagtattattttctcccatgaagacggtacgcgactgggcgtggagcatctggtcgcattgggtcaccagcaaatcgcgctgttagcgggcccattaagttctgtctcggcgcgtctgcgtctggctggctggcataaatatctcactcgcaatcaaattcagccgatagcggaacgggaaggcgactggagtgccatgtccggttttcaacaaaccatgcaaatgctgaatgagggcatcgttcccactgcgatgctggttgccaacgatcagatggcgctgggcgcaatgcgcgccattaccgagtccgggctgcgcgttggtgcggatatctcggtagtgggatacgacgataccgaagacagctcatgttatatcccgccgttaaccaccatcaaacaggattttcgcctgctggggcaaaccagcgtggaccgcttgctgcaactctctcagggccaggcggtgaagggcaatcagctgttgcccgtctcactggtgaaaagaaaaaccaccctggcgcccaatacgcaaaccgcctctccccgcgcgttggccgattcattaatgcagctggcacgacaggtttcccgactggaaagcgggcagtgagcgcaacgcaattaatgtgagttagctcactcattaggcaccccaggctttacactttatgcttccggctcgtatgttgtgtggaattgtgagcggataacaatttcacacaggaaacagctatgaccatgattacggattcactggccgtcgttttacaacgtcgtgactgggaaaaccctggcgttacccaacttaatcgccttgcagcacatccccctttcgccagctggcgtaatagcgaagaggcccgcaccgatcgcccttcccaacagttgcgcagcctgaatggcgaatggcgctttgcctggtttccggcaccagaagcggtgccggaaagctggctggagtgcgatcttcctgaggccgatactgtcgtcgtcccctcaaactggcagatgcacggttacgatgcgcccatctacaccaacgtaacctatcccattacggtcaatccgccgtttgttcccacggagaatccgacgggttgttactcgctcacatttaatgttgatgaaagctggctacaggaaggccagacgcgaattatttttgatggcgttggaatt

SEQ ID NO: 4 - protein, 383 aa, Artificial Sequence
  Synthetic GST-PTH-CBD fusion protein
MSPILGYWKIKGLVQPTRLLLEYLEEKYEEHLYERDEGDKWRNKKFELGLEFPNLPYYIDGDVKLTQSMAIIRYIADKHNMLGGCPKERAEISMLEGAVLDIRYGVSRIAYSKDFETLKVDFLSKLPEMLKMFEDRLCHKTYLNGDHVTHPDFMLYDALDVVLYMDPMCLDAFPKLVCFKKRIEAIPQIDKYLKSSKYIAWPLQGWQATFGGGDHPPKSDLIEGRSVSEIQLMHNLGKHLNSMERVEWLRKKLQDVHNGINSPVYPIGTEKEPNNSKETASGPIVPGIPVSGTIENTSDQDYFYFDVITPGEVKIDINKLGYGGATWVVYDENNNAVSYATDDGQNLSGKFKADKPGRYYIHLYMFNGSYMPYRINIEGSVGR

SEQ ID NO: 5 - protein, 4 aa, Artificial Sequence
  Synthetic peptide: Factor Xa recognition sequence
IEGR

SEQ ID NO: 6 - protein, 1021 aa, Clostridium histolyticum
MKRKCLSKRLMLAITMATIFTVNSTLPIYAAVDKNNATAAVQNESKRYTVSYLKTLNYYDLVDLLVKTEIENLPDLFQYSSDAKEFYGNKTRMSFIMDEIGRRAPQYTEIDHKGIPTLVEVVRAGFYLGFHNKELNEINKRSFKERVIPSILAIQKNPNFKLGTEVQDKIVSATGLLAGNETAPPEVVNNFTPILQDCIKNIDRYALDDLKSKALFNVLAAPTYDITEYLRATKEKPENTPWYGKIDGFINELKKLALYGKINDNNSWIIDNGIYHIAPLGKLHSNNKIGIETLTEVMKVYPYLSMQHLQSADQIKRHYDSKDAEGNKIPLDKFKKEGKEKYCPKTYTFDDGKVIIKAGARVEEEKVKRLYWASKEVNSQFFRVYGIDKPLEEGNPDDILTMVIYNSPEEYKLNSVLYGYDTNNGGMYIEPEGTFFTYEREAQESTYTLEELFRHEYTHYLQGRYAVPGQWGRTKLYDNDRLTWYEEGGAELFAGSTRTSGILPRKSIVSNIHNTTRNNRYKLSDTVHSKYGASFEFYNYACMFMDYMYNKDMGILNKLNDLAKNNDVDGYDNYIRDLSSNYALNDKYQDHMQERIDNYENLTVPFVADDYLVRHAYKNPNEIYSEISEVAKLKDAKSEVKKSQYFSTFTLRGSYTGGASKGKLEDQKAMNKFIDDSLKKLDTYSWSGYKTLTAYFTNYKVDSSNRVTYDVVFHGYLPNEGDSKNSLPYGKINGTYKGTEKEKIKFSSEGSFDPDGKIVSYEWDFGDGNKSNEENPEHSYDKVGTYTVKLKVTDDKGESSVSTTTAEIKDLSENKLPVIYMHVPKSGALNQKVVFYGKGTYDPDGSIAGYQWDFGDGSDFSSEQNPSHVYTKKGEYTVTLRVMDSSGQMSEKTMKIKITDPVYPIGTEKEPNNSKETASGPIVPGIPVSGTIENTSDQDYFYFDVITPGEVKIDINKLGYGGATWVVYDENNNAVSYATDDGQNLSGKFKADKPGRYYIHLYMFNGSYMPYRINIEGSVGR

SEQ ID NO: 7 - protein, 84 aa, Homo sapiens
SVSEIQLMHNLGKHLNSMERVEWLRKKLQDVHNFVALGAPLAPRDAGSQRPRKKEDNVLVESHEKSLGEADKADVNVLTKAKSQ

SEQ ID NO: 8 - protein, 141 aa, Homo sapiens
AVSEHQLLHDKGKSIQDLRRRFFLHHLIAEIHTAEIRATSEVSPNSKPSPNTKNHPVRFGSDDEGRYLTQETNKVETYKEQPLKTPGKKKKGKPGKRKEQEKKKRRTRSAWLDSGVTGSGLEGDHLSDTSTTSLELDSRRH

SEQ ID NO: 9 - protein, 160 aa, Artificial Sequence
  Synthetic Gly-Ser-PTH(1-33)-CBD fusion protein
GSSVSEIQLMHNLGKHLNSMERVEWLRKKLQDVHNGINSPVYPIGTEKEPNNSKETASGPIVPGIPVSGTIENTSDQDYFYFDVITPGEVKIDINKLGYGGATWVVYDENNNAVSYATDDGQNLSGKFKADKPGRYYIHLYMFNGSYMPYRINIEGSVGR

SEQ ID NO: 10 - protein, 152 aa, Artificial Sequence
  Synthetic PTH(7-33)-CBD fusion protein
LMHNLGKHLNSMERVEWLRKKLQDVHNGINSPVYPIGTEKEPNNSKETASGPIVPGIPVSGTIENTSDQDYFYFDVITPGEVKIDINKLGYGGATWVVYDENNNAVSYATDDGQNLSGKFKADKPGRYYIHLYMFNGSYMPYRINIEGSVGR

SEQ ID NO: 11 - protein, 35 aa, Artificial Sequence
  Synthetic PTH(1-33) with Gly-Ser amino terminal extension
GSSVSEIQLMHNLGKHLNSMERVEWLRKKLQDVHN

SEQ ID NO: 12 - protein, 6 aa, Artificial Sequence
  Synthetic thrombin cleavage sequence
LVPRGS

SEQ ID NO: 13 - protein, 111 aa, Clostridium histolyticum
LKEKENNDSSDKATVIPNFNTTMQGSLLGDDSRDYYSFEVKEEGEVNIELDKKDEFGVTWTLHPESNINDRITYGQVDGNKVSNKVKLRPGKYYLLVYKYSGSGNYELRVN

SEQ ID NO: 14 - protein, 111 aa, C. sporogenes
IHEKENNDSFESANKIVLNAPILGSLNGEDLRDIYSFEIKETKDLNIKLTNLNNLGLTWTLYKESDLNNYIAYGSKLGSTIVGNCHVTPGKYYLYVYKYSGNNGNYSLIIK

SEQ ID NO: 15 - protein, 111 aa, C. botulinum
IYEKENNDSFETANKIMLNTTVLGNLNGKDVRDIYSFDIKEAKDLDIKLNNLNNLGLAWNLYKESDLNNYIAYGSVSGNTIKGKCNVAPGKYYLYVYKYSGDNGNYSLAIK

SEQ ID NO: 16 - protein, 111 aa, B. cereus
LTESEPNNRPEEANRIGLNTTIKGSLIGGDHTDVYTFNVASAKNINISVLNEYGIGMTWVLHHESDMQNYAAYGQVNGNHIEANFNAKPGKYYLYVYKYDNGDGTYELSVK

SEQ ID NO: 17 - protein, 111 aa, B. anthracis
LTESEPNNRPEEANRIGLNTTIKGSLIGGDHTDVYTFNVASAKNIDISVLNEYGIGMTWVLHHESDMQNYAAYGQANGNHIEANFNAKPGKYYLYVYKYDNGDGTYELSVK

SEQ ID NO: 18 - protein, 111 aa, Bacillus sp.
KTEIEPNNRPEEATMLPFNTPLSGSLMEDDHTDVYEFNVTSPKEIDISVLNENQIGMTWVLYHESDSQNYASFGQEDGNMINGKWNAKPGKYYLYVYKFENENGTYTVHVQ

SEQ ID NO: 19 - protein, 111 aa, L. sphaericus
KAEIEPNNRPEEATILPFNTPLKGRLMDDDHTDVYEFNVTSPKELDISVLNENRIGMTWVLYHESDSQNYASFGQEEGNMINGKLHAEPGKYYLYVYKFENENGTYTVQVQ

SEQ ID NO: 20 - protein, 111 aa, C. cerus
VTENEPNNEPRQANKVNFHTPVKGTLHNSDRVDVFTFQIDSPENINISLLNEQNIGMTWVLHHESDLNNYVAYGENEGNVVKGTYNAKPGKYYLYVYKYENKDGSYVLNIK

SEQ ID NO: 21 - protein, 111 aa, B. mycoides
SVEKEPNNSFQTANKLQLNQLLRASLGNGDTSDYFEINVETARNLQINVTKENNIGVNWVLYSAADLNNYVTYAQTQGNKLVGSYNAHPGKYYLHVYQYGGGTGNYTVEVK

SEQ ID NO: 22 - protein, 112 aa, B. weihensteph
AVEKEPNNSFDAANPLSLNALLRGNLSDQDQVDRFVIDVKDPKDLQITVTNEQNLGLNWVLYSESDLNNYVTYATKRDGNKLLGNYNAKPGKYYLSVYKYGGGTGNFTVEVK

SEQ ID NO: 23 - protein, 111 aa, B. brevis
EKEQEPNNSFSEANPLKSNVELSGQTSKQDDKDIFALKVLGNGTVKINVTSEHDTGLNWVVHHEDDLNNYLAYPKTSGKTLSGEFEATPGTYYLSVYNFNGETIPYKVTAE

SEQ ID NO: 24 - protein, 111 aa, B. brevis
PTEVEPNNSFDDANTLQLGKEISGQTDRTDDKDTYMIQVEEEGVIQVTVSSEKDEGLNWVVFHEDDLKTYFAYPKTTGKKLTGEFEAKPGKYYLLVYNTNNTKIPYKAIVN

SEQ ID NO: 25 - protein, 112 aa, C. perfringens
IKEVENNNDFDKAMKVDSNSKIVGTLSNDDLKDIYSIDIKNPSDLNIVVENLDNIKMNWLLYSADDLSNYVDYANADGNKLSNTCKLNPGKYYLCVYQFENSGTGNYTVNLQ

SEQ ID NO: 26 - protein, 115 aa, C. sporogenes
ISEKEDNDSFDKANRVGKNQTVLATLDTKDNRDTYYFDALAARTIDIVMENTDNNSTIFNWLAYSSDNTNNYIGYPTKKEGNKLMGSFKVPKPGRYYILAYKNSSNKINYKLTIN

SEQ ID NO: 27 - protein, 115 aa, C. botulinum
ISEKEDNNSFDKANRVCKNQSVIATLDTNDPRDTYYFDALTAGNIEVTMGNTDNSSNEFNWLAYSSDNTNNYIGYATKREGNKITGNFKVDKPGRYYIVAYKTSSNKINYKLNIK

SEQ ID NO: 28 - protein, 115 aa, C. sporogenes
VSEKEDNNDFTTANPVYYKDLVNGSVSSSDNKDTFYFTVTKPSDITITVEKTNNDKSEFNWLLFSDEDKSNYMAFPNKELGNQLSNTVKINKPGKYYLVIYKTLGEKVDYKFSIE

SEQ ID NO: 29 - protein, 115 aa, C. botulinum
VSEKENNNDYVNANPVYSKDLVNGSVSSSDDRDIFYFNVTKPSDITINVEKINKDKSEFSWLLFSEEDKSNYITYPNKELENLFYSTVKIDKPGKYYLVIYKVSGEKSDYRFNIE

SEQ ID NO: 30 - protein, 113 aa, C. sordellii
GVEQEDNNSFEKANPFSINQLVKGELDNNKDTSDYFKFEVKEDAQLNISLEKTEGDGVNWLLFKDSDLENYIASPTESIDNKLNGKVDLKVGTYYLEVYGYGSSPVKYNFKVT

SEQ ID NO: 31 - protein, 113 aa, Clostridium histolyticum
TKEMEPNDDIKEANGPIVEGVTVKGDLNGSDDADTFYFDVKEDGDVTIELPYSGSSNFTWLVYKEGDDQNHIASGIDKNNSKVGTFKSTKGRHYVFIYKHDSASNISYSLNIK

SEQ ID NO: 32 - protein, 113 aa, C. perfringens
INESEPNNDFEKANQIAKSNMLVKGTLSEEDYSDKYYFDVAKKGNVKITLNNLNSVGITWTLYKEGDLNNYVLYATGNEGTVLKGEKTLEPGRYYLSVYTYDNQSGAYTVNVK

SEQ ID NO: 33 - protein, 113 aa, C. sordellii
SQEVGNDDTFETANGPIKINTNYSGDLSDTDNKDYYYFNLDNPSNINITLENLDNKGISWQLFHESDLNNYVAYPTTSGAILNGDYNATKPGKYYILVYNHDKSIANYNLKVN

SEQ ID NO: 34 - protein, 111 aa, Clostridium histolyticum
GTEKEPNNSKETASGPIVPGIPVSGTIENTSDQDYFYFDVITPGEVKIDINKLGYGGATWVVYDENNNAVSYATDDGQNLSGKFKADKPGRYYIHLYMFNGSYMPYRINIE

SEQ ID NO: 35 - protein, 30 aa, Artificial Sequence
  Synthetic peptide
  misc_feature (1)..(30): Any Xaa is hydroxyproline
PXGPXGPXGPXGPXGPXGPXGPXGPXGPXG

SEQ ID NO: 36 - protein, 30 aa, Artificial Sequence
  Synthetic peptide
  misc_feature (1)..(30): Any Xaa is hydroxyproline
PXGPXGPXGPXGPXGPXGPXAPXGPXGPXG

SEQ ID NO: 37 - protein, 30 aa, Artificial Sequence
  Synthetic peptide
  misc_feature (1)..(30): Any Xaa is hydroxyproline
PXGPXGPXGPXGPXGPXAPXGPXGPXGPXG

SEQ ID NO: 38 - protein, 30 aa, Artificial Sequence
  Synthetic peptide
  misc_feature (1)..(30): Any Xaa is hydroxyproline
PXGPXGPXGPXGPXAPXGPXGPXGPXGPXG

SEQ ID NO: 39 - protein, 30 aa, Artificial Sequence
  Synthetic peptide
  misc_feature (1)..(30): Any Xaa is hydroxyproline
PXGPXGPXGPXAPXGPXGPXGPXGPXGPXG

SEQ ID NO: 40 - protein, 24 aa, Artificial Sequence
  Synthetic peptide
  misc_feature (1)..(24): Any Xaa is hydroxyproline
PXGPXGPXGPCGPXGPXGPXGPXG

SEQ ID NO: 41 - protein, 31 aa, Artificial Sequence
  Synthetic peptide
  misc_feature (1)..(31): Any Xaa is hydroxyproline
PXGPXGPXGPXGPXAPXGPXGPXGPXGPXGC

SEQ ID NO: 42 - protein, 22 aa, Artificial Sequence
  Synthetic peptide
  misc_feature (1)..(22): Any Xaa is hydroxyproline
GPXGPXGPXGPXGPXGPXGPXG

SEQ ID NO: 43 - protein, 31 aa, Artificial Sequence
  Synthetic peptide
  misc_feature (1)..(31): Any Xaa is hydroxyproline
GPXGPXGPXGPXGPXGPXGPXGPRGPRGPRG

SEQ ID NO: 44 - protein, 9 aa, Artificial Sequence
  Synthetic peptide
  misc_feature (1)..(9): Any Xaa is hydroxyproline
PXGPXGPXG

SEQ ID NO: 45 - protein, 9 aa, Artificial Sequence
  Synthetic peptide
  misc_feature (1)..(9): Any Xaa is hydroxyproline
PXGPXGPXA

SEQ ID NO: 46 - protein, 26 aa, Artificial Sequence
  Synthetic peptide
  misc_feature (1)..(26): Any Xaa is hydroxyproline
GPRGPXGPXGPXGPXGPXGPXGPXGC

SEQ ID NO: 47 - protein, 7 aa, Artificial Sequence
  Synthetic peptide: GST Tag
GSPGIPG